European Patent Specification EP 3 692 014 B1, published November 22, 2023. Title: PROBE FOR SELECTIVELY CHARACTERIZING ENZYMES INVOLVED IN XENOBIOTIC METABOLISM AND METHOD OF MAKING AND USING THE SAME. Applicant: Battelle Memorial Institute Wright, Aaron   T. Ramos-Hunter, Susan Whidbey, Christopher. The sequence listing filed with the application follows.

SEQUENCE LISTING (4 sequences)

SEQ ID NO: 1 - DNA, 43 bp, Artificial Sequence
  uidA_F primer
aactttaagaaggagatataatgttacgtcctgtagaaacccc

SEQ ID NO: 2 - DNA, 59 bp, Artificial Sequence
  uidA_R primer
ttgttagcagccggatctcattaatggtgatggtgatggtgttgtttgcctccctgctg

SEQ ID NO: 3 - DNA, 39 bp, Artificial Sequence
  pET_F primer
caccatcaccatcaccattaatgagatccggctgctaac

SEQ ID NO: 4 - DNA, 58 bp, Artificial Sequence
  pET_R primer
tatatctccttcttaaagttaaacaaaattatttctagaggggaattgttatccgctc